European Patent Application EP 4 257 604 A1, published October 11, 2023. Title: ANTI-TSLP ANTIBODY PHARMACEUTICAL COMPOSITION AND USE THEREOF. Applicant: Jiangsu Hengrui Pharmaceuticals Co., Ltd. Shanghai Hengrui Pharmaceutical Co., Ltd. Application PCT/CN2021/132037. The sequence listing filed with the application follows.

SEQUENCE LISTING (146 sequences)

SEQ ID NO: 1 - protein, 176 aa, Artificial Sequence
  huTSLP-his
MFPFALLYVLSVSFRKIFILQLVGLVLTYDFTNCDFEKIKAAYLSTISKDLITYMSGTKSTEFNNTVSCSNRPHCLTEIQSLTFNPTAGCASLAKEMFAMKTKAALAIWCPGYSETQINATQAMKKARKSKVTTNKCLEQVSQLQGLWRRFNRPLLKQQGSSDYKDDDDKHHHHHH

SEQ ID NO: 2 - protein, 398 aa, Artificial Sequence
  huTSLP-Fc
MFPFALLYVLSVSFRKIFILQLVGLVLTYDFTNCDFEKIKAAYLSTISKDLITYMSGTKSTEFNNTVSCSNRPHCLTEIQSLTFNPTAGCASLAKEMFAMKTKAALAIWCPGYSETQINATQAMKKARKSKVTTNKCLEQVSQLQGLWRRFNRPLLKQQDIEGRMDEPKSSDKTHTCPPCPAPELLGGPSVFLFPPKPKDTLMISRTPEVTCVVVDVSHEDPEVKFNWYVDGVEVHNAKTKPREEQYNSTYRVVSVLTVLHQDWLNGKEYKCKVSNKALPAPIEKTISKAKGQPREPQVYTLPPSRDELTKNQVSLTCLVKGFYPSDIAVEWESNGQPENNYKTTPPVLDSDGSFFLYSKLTVDKSRWQQGNVFSCSVMHEALHNHYTQKSLSLSPGK

SEQ ID NO: 3 - protein, 168 aa, Artificial Sequence
  cynoTSLP-His
METDTLLLWVLLLWVPGSTGYDFTNCDFQKIEADYLRTISKDLITYMSGTKSTDFNNTVSCSNRPHCLTEIQSLTFNPTPRCASLAKEMFARKTKATLALWCPGYSETQINATQAMKKARKSKVTTNKCLEQVSQLLGLWRRFIRTLLKQQGSSDYKDDDDKHHHHHH

SEQ ID NO: 4 - protein, 390 aa, Artificial Sequence
  cyno TSLP-Fc
METDTLLLWVLLLWVPGSTGYDFTNCDFQKIEADYLRTISKDLITYMSGTKSTDFNNTVSCSNRPHCLTEIQSLTFNPTPRCASLAKEMFARKTKATLALWCPGYSETQINATQAMKKARKSKVTTNKCLEQVSQLLGLWRRFIRTLLKQQDIEGRMDEPKSSDKTHTCPPCPAPELLGGPSVFLFPPKPKDTLMISRTPEVTCVVVDVSHEDPEVKFNWYVDGVEVHNAKTKPREEQYNSTYRVVSVLTVLHQDWLNGKEYKCKVSNKALPAPIEKTISKAKGQPREPQVYTLPPSRDELTKNQVSLTCLVKGFYPSDIAVEWESNGQPENNYKTTPPVLDSDGSFFLYSKLTVDKSRWQQGNVFSCSVMHEALHNHYTQKSLSLSPGK

SEQ ID NO: 5 - protein, 446 aa, Artificial Sequence
  TSLPR-Fc-ECD
GAAEGVQIQIIYFNLETVQVTWNASKYSRTNLTFHYRFNGDEAYDQCTNYLLQEGHTSGCLLDAEQRDDILYFSIRNGTHPVFTASRWMVYYLKPSSPKHVRFSWHQDAVTVTCSDLSYGDLLYEVQYRSPFDTEWQSKQENTCNVTIEGLDAEKCYSFWVRVKAMEDVYGPDTYPSDWSEVTCWQRGEIRDACAETPTPPKPKLSKDIEGRMDEPKSSDKTHTCPPCPAPELLGGPSVFLFPPKPKDTLMISRTPEVTCVVVDVSHEDPEVKFNWYVDGVEVHNAKTKPREEQYNSTYRVVSVLTVLHQDWLNGKEYKCKVSNKALPAPIEKTISKAKGQPREPQVYTLPPSRDELTKNQVSLTCLVKGFYPSDIAVEWESNGQPENNYKTTPPVLDSDGSFFLYSKLTVDKSRWQQGNVFSCSVMHEALHNHYTQKSLSLSPGK

SEQ ID NO: 6 - protein, 121 aa, Mus musculus
EVQLQQSGPVLVKPGASVKMSCKASGYTFTDDYMNWVKQSHGKSLEWIGIISPYNGGTSYNQKFKGKATLTVDKSSSTAYMELNSLTSEDSAVYYCAREDYDYDGYAMDHWGQGTSVTVSS

SEQ ID NO: 7 - protein, 105 aa, Mus musculus
QIVLSQSPAILSASPGEKVTMTCRASSSVSYMHWYQQKPGSSPKPWIYATSNLASGVPARFSGSGSGTSYSLTISRVEAEDAATYYCQQWSSNRTFGGGTKLEIK

SEQ ID NO: 8 - protein, 120 aa, Mus musculus
QAYLQQSGAELVRPGASVKMSCKASGFAFTTYNMHWVKHTPGQGLEWIGAIYPGNGETSYNQKFKDRATLTVDKSSRTAYMQLSSLTSEDSAVYFCAREDDYGEGYFDVWGAGTTVTVSS

SEQ ID NO: 9 - protein, 111 aa, Mus musculus
DIVLTQSPASLAVSLGQRATISCRASESVDNSGLSFMHWYQQKPGQPPRLLLYRASNLGSGIPARFSGSGSGTDFTLTLNPVETDDVATYYCQQINTDPLTFGAGTKLELK

SEQ ID NO: 10 - protein, 119 aa, Mus musculus
QVQLQQSGAELVRPGTSVKVSCKASGYAFTNYLIEWVKQRPGQGLEWIGVIDPGNGDTNYNENFKGKATLTADKSSSTAYIELSRLTSEDSAVYFCAREDNTGTAFDYWGQGTTLTVSS

SEQ ID NO: 11 - protein, 107 aa, Mus musculus
SIVMTQTPKFLLVSAGDRVTISCKASQSVSSDVTWYQQKPGQSPKLLIYYVSNHYTGVPDRFTGSGYGTDFTFTISSVQAEDLAVYFCQQHHRFPLTFGAGTKLELK

SEQ ID NO: 12 - protein, 117 aa, Mus musculus
QVQLQQSGPQLVRPGASVKISCKASGYSFTTYWMHWVKQRPGQGLEWIGMIDPSDSETTLIQKFKDKATLTVDKSSSTAYMQLSSPTSEDSAVYYCARTLDGYYDYWGQGTTLTVSS

SEQ ID NO: 13 - protein, 107 aa, Mus musculus
DIQMTQSPASLSASVGETVTITCRASENIYSYLAWYQQKQGKSPQLLVYFAKTLAEGVPSRFSGSVSGTQFSLKINSLQPEDFGSYYCQHHYGTPWTFGGGTKLEIK

SEQ ID NO: 14 - protein, 5 aa, Mus musculus
DDYMN

SEQ ID NO: 15 - protein, 17 aa, Mus musculus
IISPYNGGTSYNQKFKG

SEQ ID NO: 16 - protein, 12 aa, Mus musculus
EDYDYDGYAMDH

SEQ ID NO: 17 - protein, 10 aa, Mus musculus
RASSSVSYMH

SEQ ID NO: 18 - protein, 7 aa, Mus musculus
ATSNLAS

SEQ ID NO: 19 - protein, 8 aa, Mus musculus
QQWSSNRT

SEQ ID NO: 20 - protein, 5 aa, Mus musculus
TYNMH

SEQ ID NO: 21 - protein, 17 aa, Mus musculus
AIYPGNGETSYNQKFKD

SEQ ID NO: 22 - protein, 11 aa, Mus musculus
EDDYGEGYFDV

SEQ ID NO: 23 - protein, 15 aa, Mus musculus
RASESVDNSGLSFMH

SEQ ID NO: 24 - protein, 7 aa, Mus musculus
RASNLGS

SEQ ID NO: 25 - protein, 9 aa, Mus musculus
QQINTDPLT

SEQ ID NO: 26 - protein, 5 aa, Mus musculus
NYLIE

SEQ ID NO: 27 - protein, 17 aa, Mus musculus
VIDPGNGDTNYNENFKG

SEQ ID NO: 28 - protein, 10 aa, Mus musculus
EDNTGTAFDY

SEQ ID NO: 29 - protein, 11 aa, Mus musculus
KASQSVSSDVT

SEQ ID NO: 30 - protein, 7 aa, Mus musculus
YVSNHYT

SEQ ID NO: 31 - protein, 9 aa, Mus musculus
QQHHRFPLT

SEQ ID NO: 32 - protein, 5 aa, Mus musculus
TYWMH

SEQ ID NO: 33 - protein, 17 aa, Mus musculus
MIDPSDSETTLIQKFKD

SEQ ID NO: 34 - protein, 8 aa, Mus musculus
TLDGYYDY

SEQ ID NO: 35 - protein, 11 aa, Mus musculus
RASENIYSYLA

SEQ ID NO: 36 - protein, 7 aa, Mus musculus
FAKTLAE

SEQ ID NO: 37 - protein, 9 aa, Mus musculus
QHHYGTPWT

SEQ ID NO: 38 - protein, 105 aa, Artificial Sequence
  hu3 VL-CDR grafted
EIVLTQSPATLSLSPGERATLSCRASSSVSYMHWYQQKPGQAPRLLIYATSNLASGIPARFSGSGSGTDFTLTISRLEPEDFAVYYCQQWSSNRTFGGGTKVEIK

SEQ ID NO: 39 - protein, 105 aa, Artificial Sequence
  hu3VL2
EIVLTQSPATLSLSPGERATLSCRASSSVSYMHWYQQKPGQAPRPLIYATSNLASGIPARFSGSGSGTDYTLTISRLEPEDFAVYYCQQWSSNRTFGGGTKVEIK

SEQ ID NO: 40 - protein, 105 aa, Artificial Sequence
  hu3VL3
EIVLTQSPATLSLSPGERATLSCRASSSVSYMHWYQQKPGQAPRPWIYATSNLASGVPARFSGSGSGTDYTLTISRLEPEDFAVYYCQQWSSNRTFGGGTKVEIK

SEQ ID NO: 41 - protein, 105 aa, Artificial Sequence
  hu3VL4
EIVLTQSPATLSLSPGERATLSCRASSSVSYMHWYQQKPGQAPRPWIYATSNLASGVPARFSGSGSGTSYTLTISRLEPEDFAVYYCQQWSSNRTFGGGTKVEIK

SEQ ID NO: 42 - protein, 121 aa, Artificial Sequence
  hu3VH1
EVQLVQSGAEVKKPGASVKVSCKASGYTFTDDYMNWVRQAPGQRLEWMGIISPYNGGTSYNQKFKGRVTITRDTSASTAYMELSSLRSEDTAVYYCAREDYDYDGYAMDHWGQGTTVTVSS

SEQ ID NO: 43 - protein, 121 aa, Artificial Sequence
  hu3VH2
EVQLVQSGAEVKKPGASVKVSCKASGYTFTDDYMNWVRQAPGQRLEWMGIISPYNGGTSYNQKFKGRVTLTVDKSASTAYMELSSLRSEDTAVYYCAREDYDYDGYAMDHWGQGTTVTVSS

SEQ ID NO: 44 - protein, 121 aa, Artificial Sequence
  hu3VH3
EVQLVQSGAEVKKPGASVKVSCKASGYTFTDDYMNWVKQAPGQRLEWIGIISPYNGGTSYNQKFKGRATLTVDKSASTAYMELSSLRSEDTAVYYCAREDYDYDGYAMDHWGQGTTVTVSS

SEQ ID NO: 45 - protein, 12 aa, Artificial Sequence
  hu3 HCDR3-H110Y
EDYDYDGYAMDY

SEQ ID NO: 46 - protein, 8 aa, Artificial Sequence
  hu3LCDR3-N93D
QQWSSDRT

SEQ ID NO: 47 - protein, 12 aa, Artificial Sequence
  hu3 HCDR3
  DOMAIN (12)..(12): Xaa is selected from the group consisting of His and Tyr
EDYDYDGYAMDX

SEQ ID NO: 48 - protein, 8 aa, Artificial Sequence
  hu3 LCDR3(1
  DOMAIN (6)..(6): Xaa is selected from the group consisting of Asn and Asp
QQWSSXRT

SEQ ID NO: 49 - protein, 105 aa, Artificial Sequence
  hu3VL4-N93D
EIVLTQSPATLSLSPGERATLSCRASSSVSYMHWYQQKPGQAPRPWIYATSNLASGVPARFSGSGSGTSYTLTISRLEPEDFAVYYCQQWSSDRTFGGGTKVEIK

SEQ ID NO: 50 - protein, 121 aa, Artificial Sequence
  hu3VH2-H110Y
EVQLVQSGAEVKKPGASVKVSCKASGYTFTDDYMNWVRQAPGQRLEWMGIISPYNGGTSYNQKFKGRVTLTVDKSASTAYMELSSLRSEDTAVYYCAREDYDYDGYAMDYWGQGTTVTVSS

SEQ ID NO: 51 - protein, 105 aa, Artificial Sequence
  hu3VL5
EIVLTQSPATLSLSPGERATLSCRASSSVSYMHWYQQKPGQAPRPWIYATSNLASGVPARFSGSGSGTSYTLTISRLEPEDFAVYYCQQSDNVRGFGGGTKVEIK

SEQ ID NO: 52 - protein, 105 aa, Artificial Sequence
  hu3VL6
EIVLTQSPATLSLSPGERATLSCRASSSVSYMHWYQQKPGQAPRPWIYATSNLASGVPARFSGSGSGTSYTLTISRLEPEDFAVYYCQQSDSGREFGGGTKVEIK

SEQ ID NO: 53 - protein, 8 aa, Artificial Sequence
  hu3 LCDR-V1
QQSDNVRG

SEQ ID NO: 54 - protein, 8 aa, Artificial Sequence
  hu3 LCDR3-V2
QQSDSGRE

SEQ ID NO: 55 - protein, 8 aa, Artificial Sequence
  hu3 LCDR3(2)
  DOMAIN (5)..(5): Xaa is selected from the group consisting of Asn and Ser
  DOMAIN (6)..(6): Xaa is selected from the group consisting of Val and Gly
  DOMAIN (8)..(8): Xaa is selected from the group consisting of Gly and Glu
QQSDXXRX

SEQ ID NO: 56 - protein, 111 aa, Artificial Sequence
  hu119-VL grafted(IGKV4-1*01)
DIVMTQSPDSLAVSLGERATINCRASESVDNSGLSFMHWYQQKPGQPPKLLIYRASNLGSGVPDRFSGSGSGTDFTLTISSLQAEDVAVYYCQQINTDPLTFGQGTKLEIK

SEQ ID NO: 57 - protein, 111 aa, Artificial Sequence
  hu119VL2
DIVLTQSPDSLAVSLGERATINCRASESVDNSGLSFMHWYQQKPGQPPKLLIYRASNLGSGVPDRFSGSGSGTDFTLTISSLQAEDVAVYYCQQINTDPLTFGQGTKLEIK

SEQ ID NO: 58 - protein, 111 aa, Artificial Sequence
  hu119VL3
DIVMTQSPDSLAVSLGERATINCRASESVDNSGLSFMHWYQQKPGQPPKLLLYRASNLGSGIPDRFSGSGSGTDFTLTISSLQAEDVAVYYCQQINTDPLTFGQGTKLEIK

SEQ ID NO: 59 - protein, 111 aa, Artificial Sequence
  hu119VL4 (Grafted, IGKV3-11*01)
EIVLTQSPATLSLSPGERATLSCRASESVDNSGLSFMHWYQQKPGQAPRLLIYRASNLGSGIPARFSGSGSGTDFTLTISSLEPEDFAVYYCQQINTDPLTFGQGTKLEIK

SEQ ID NO: 60 - protein, 111 aa, Artificial Sequence
  hu119VL5
EIVLTQSPATLSLSPGERATLSCRASESVDNSGLSFMHWYQQKPGQPPRLLLYRASNLGSGIPARFSGSGSGTDFTLTISSLEPEDFAVYYCQQINTDPLTFGQGTKLEIK

SEQ ID NO: 61 - protein, 111 aa, Artificial Sequence
  hu119VL6
DIVLTQSPATLSLSPGERATLSCRASESVDNSGLSFMHWYQQKPGQPPRLLLYRASNLGSGIPARFSGSGSGTDFTLTISSLEPEDFAVYYCQQINTDPLTFGQGTKLEIK

SEQ ID NO: 62 - protein, 120 aa, Artificial Sequence
  hu119VH1 (Grafted)
EVQLVQSGAEVKKPGSSVKVSCKASGGTFSTYNMHWVRQAPGQGLEWMGAIYPGNGETSYNQKFKDRVTITADKSTSTAYMELSSLRSEDTAVYYCAREDDYGEGYFDVWGQGTTVTVSS

SEQ ID NO: 63 - protein, 120 aa, Artificial Sequence
  hu119VH2
EVQLVQSGAEVKKPGSSVKVSCKASGFTFSTYNMHWVRQAPGQGLEWMGAIYPGNGETSYNQKFKDRVTLTVDKSTSTAYMELSSLRSEDTAVYYCAREDDYGEGYFDVWGQGTTVTVSS

SEQ ID NO: 64 - protein, 120 aa, Artificial Sequence
  hu119VH3
EVQLVQSGAEVKKPGSSVKVSCKASGFTFSTYNMHWVKHAPGQGLEWIGAIYPGNGETSYNQKFKDRATLTVDKSTSTAYMELSSLRSEDTAVYYCAREDDYGEGYFDVWGQGTTVTVSS

SEQ ID NO: 65 - protein, 120 aa, Artificial Sequence; identical to SEQ ID NO: 64
  hu119VH4

SEQ ID NO: 66 - protein, 120 aa, Artificial Sequence
  hu119VH5
EVQLVQSGAEVKKPGSSVKVSCKASGGTFSTYNMHWVRQAPGQGLEWIGAIYPGNGETSYNQKFKDRATLTVDKSTSTAYMELSSLRSEDTAVYYCAREDDYGEGYFDVWGQGTTVTVSS

SEQ ID NO: 67 - protein, 120 aa, Artificial Sequence
  hu119VH6
EAQLVQSGAEVKKPGSSVKVSCKASGFTFSTYNMHWVRQAPGQGLEWIGAIYPGNGETSYNQKFKDRATLTVDKSTSTAYMELSSLRSEDTAVYYCAREDDYGEGYFDVWGQGTTVTVSS

SEQ ID NO: 68 - protein, 120 aa, Artificial Sequence
  hu119VH7
EVQLVQSGAEVKKPGSSVKVSCKASGGTFSTYNMHWVRQAPGQGLEWIGAIYPGNGETSYNQKFKDRATLTVDKSTRTAYMELSSLRSEDTAVYYCAREDDYGEGYFDVWGQGTTVTVSS

SEQ ID NO: 69 - protein, 120 aa, Artificial Sequence
  hu119VH8
EAQLVQSGAEVKKPGSSVKVSCKASGFTFSTYNMHWVRQAPGQGLEWIGAIYPGNGETSYNQKFKDRATLTVDKSTRTAYMELSSLRSEDTAVYYCAREDDYGEGYFDVWGQGTTVTVSS

SEQ ID NO: 70 - protein, 15 aa, Artificial Sequence
  hu119 LCDR1-N31S
RASESVDSSGLSFMH

SEQ ID NO: 71 - protein, 15 aa, Artificial Sequence
  hu119 LCDR1-N31Q
RASESVDQSGLSFMH

SEQ ID NO: 72 - protein, 111 aa, Artificial Sequence
  hu119VL2-N31S
DIVLTQSPDSLAVSLGERATINCRASESVDSSGLSFMHWYQQKPGQPPKLLIYRASNLGSGVPDRFSGSGSGTDFTLTISSLQAEDVAVYYCQQINTDPLTFGQGTKLEIK

SEQ ID NO: 73 - protein, 111 aa, Artificial Sequence
  hu119VL2-N31Q
DIVLTQSPDSLAVSLGERATINCRASESVDQSGLSFMHWYQQKPGQPPKLLIYRASNLGSGVPDRFSGSGSGTDFTLTISSLQAEDVAVYYCQQINTDPLTFGQGTKLEIK

SEQ ID NO: 74 - protein, 111 aa, Artificial Sequence
  hu119VL6-N31S
DIVLTQSPATLSLSPGERATLSCRASESVDSSGLSFMHWYQQKPGQPPRLLLYRASNLGSGIPARFSGSGSGTDFTLTISSLEPEDFAVYYCQQINTDPLTFGQGTKLEIK

SEQ ID NO: 75 - protein, 111 aa, Artificial Sequence
  hu119VL6-N31Q
DIVLTQSPATLSLSPGERATLSCRASESVDQSGLSFMHWYQQKPGQPPRLLLYRASNLGSGIPARFSGSGSGTDFTLTISSLEPEDFAVYYCQQINTDPLTFGQGTKLEIK

SEQ ID NO: 76 - protein, 15 aa, Artificial Sequence
  hu119 LCDR1-
  DOMAIN (8)..(8): Xaa is selected from the group consisting of Asn, Ser, and Gln
RASESVDXSGLSFMH

SEQ ID NO: 77 - protein, 107 aa, Artificial Sequence
  hu179VL1 (Grafted (IGKV4-1*01))
DIVMTQSPDSLAVSLGERATINCKASQSVSSDVTWYQQKPGQPPKLLIYYVSNHYTGVPDRFSGSGSGTDFTLTISSLQAEDVAVYYCQQHHRFPLTFGQGTKLEIK

SEQ ID NO: 78 - protein, 107 aa, Artificial Sequence
  hu179VL2
DIVMTQSPDSLAVSLGERATINCKASQSVSSDVTWYQQKPGQSPKLLIYYVSNHYTGVPDRFSGSGSGTDFTLTISSLQAEDVAVYYCQQHHRFPLTFGQGTKLEIK

SEQ ID NO: 79 - protein, 107 aa, Artificial Sequence
  hu179 VL3
DIVMTQSPDSLAVSLGERATINCKASQSVSSDVTWYQQKPGQSPKLLIYYVSNHYTGVPDRFSGSGSGTDFTFTISSLQAEDVAVYYCQQHHRFPLTFGQGTKLEIK

SEQ ID NO: 80 - protein, 107 aa, Artificial Sequence
  hu179 VL4
SIVMTQSPDSLAVSLGERATINCKASQSVSSDVTWYQQKPGQSPKLLIYYVSNHYTGVPDRFSGSGSGTDFTLTISSLQAEDVAVYYCQQHHRFPLTFGQGTKLEIK

SEQ ID NO: 81 - protein, 107 aa, Artificial Sequence
  hu179VL5Grafted(IGKV2-29*02)
DIVMTQTPLSLSVTPGQPASISCKASQSVSSDVTWYLQKPGQSPQLLIYYVSNHYTGVPDRFSGSGSGTDFTLKISRVEAEDVGVYYCQQHHRFPLTFGQGTKLEIK

SEQ ID NO: 82 - protein, 107 aa, Artificial Sequence
  hu179VL6
SIVMTQTPLSLSVTPGQPASISCKASQSVSSDVTWYLQKPGQSPQLLIYYVSNHYTGVPDRFSGSGSGTDFTLKISRVEAEDVGVYYCQQHHRFPLTFGQGTKLEIK

SEQ ID NO: 83 - protein, 107 aa, Artificial Sequence
  hu179VL7
SIVMTQTPLSLSVTPGQPASISCKASQSVSSDVTWYLQKPGQSPQLLIYYVSNHYTGVPDRFSGSGSGTDFTFKISRVEAEDVGVYYCQQHHRFPLTFGQGTKLEIK

SEQ ID NO: 84 - protein, 107 aa, Artificial Sequence
  hu179VL8
SIVMTQTPLSLSVTPGQPASISCKASQSVSSDVTWYLQKPGQSPQLLIYYVSNHYTGVPDRFSGSGYGTDFTLKISRVEAEDVGVYYCQQHHRFPLTFGQGTKLEIK

SEQ ID NO: 85 - protein, 119 aa, Artificial Sequence
  hu179VH1Grafted
EVQLVQSGAEVKKPGSSVKVSCKASGGTFSNYLIEWVRQAPGQGLEWMGVIDPGNGDTNYNENFKGRVTITADKSTSTAYMELSSLRSEDTAVYYCAREDNTGTAFDYWGQGTTVTVSS

SEQ ID NO: 86 - protein, 119 aa, Artificial Sequence
  hu179VH2
EVQLVQSGAEVKKPGSSVKVSCKASGYTFSNYLIEWVRQAPGQGLEWMGVIDPGNGDTNYNENFKGRVTLTADKSTSTAYMELSSLRSEDTAVYYCAREDNTGTAFDYWGQGTTVTVSS

SEQ ID NO: 87 - protein, 119 aa, Artificial Sequence
  hu179VH3
EVQLVQSGAEVKKPGSSVKVSCKASGYTFSNYLIEWVRQAPGQGLEWIGVIDPGNGDTNYNENFKGRATLTADKSTSTAYIELSSLRSEDTAVYYCAREDNTGTAFDYWGQGTTVTVSS

SEQ ID NO: 88 - protein, 119 aa, Artificial Sequence
  hu179VH4
EVQLVQSGAEVKKPGSSVKVSCKASGYTFSNYLIEWVKQAPGQGLEWIGVIDPGNGDTNYNENFKGKATLTADKSTSTAYIELSRLRSEDTAVYYCAREDNTGTAFDYWGQGTTVTVSS

SEQ ID NO: 89 - protein, 119 aa, Artificial Sequence
  hu179VH5
EVQLVQSGAEVKKPGSSVKVSCKASGYAFSNYLIEWVRQAPGQGLEWIGVIDPGNGDTNYNENFKGRATLTADKSTSTAYMELSSLRSEDTAVYYCAREDNTGTAFDYWGQGTTVTVSS

SEQ ID NO: 90 - protein, 119 aa, Artificial Sequence
  hu179VH1-N55Q
EVQLVQSGAEVKKPGSSVKVSCKASGGTFSNYLIEWVRQAPGQGLEWMGVIDPGQGDTNYNENFKGRVTITADKSTSTAYMELSSLRSEDTAVYYCAREDNTGTAFDYWGQGTTVTVSS

SEQ ID NO: 91 - protein, 119 aa, Artificial Sequence
  hu179VH1-N55V
EVQLVQSGAEVKKPGSSVKVSCKASGGTFSNYLIEWVRQAPGQGLEWMGVIDPGVGDTNYNENFKGRVTITADKSTSTAYMELSSLRSEDTAVYYCAREDNTGTAFDYWGQGTTVTVSS

SEQ ID NO: 92 - protein, 119 aa, Artificial Sequence
  hu179VH1-G56V
EVQLVQSGAEVKKPGSSVKVSCKASGGTFSNYLIEWVRQAPGQGLEWMGVIDPGNVDTNYNENFKGRVTITADKSTSTAYMELSSLRSEDTAVYYCAREDNTGTAFDYWGQGTTVTVSS

SEQ ID NO: 93 - protein, 17 aa, Artificial Sequence
  hu179 HCDR2-N55Q
VIDPGQGDTNYNENFKG

SEQ ID NO: 94 - protein, 17 aa, Artificial Sequence
  hu179 HCDR2-N55V
VIDPGVGDTNYNENFKG

SEQ ID NO: 95 - protein, 17 aa, Artificial Sequence
  hu179 HCDR2-G56V
VIDPGNVDTNYNENFKG

SEQ ID NO: 96 - protein, 13 aa, Artificial Sequence
  hu179 HCDR2
  DOMAIN (6)..(6): Xaa is selected from the group consisting of Asn, Gln, and Val
  DOMAIN (7)..(7): Xaa is selected from the group consisting of Gly and Val
VIDPGXXDTNYNE

SEQ ID NO: 97 - protein, 119 aa, Artificial Sequence
  hu179VH3-N55V
EVQLVQSGAEVKKPGSSVKVSCKASGYTFSNYLIEWVRQAPGQGLEWIGVIDPGVGDTNYNENFKGRATLTADKSTSTAYIELSSLRSEDTAVYYCAREDNTGTAFDYWGQGTTVTVSS

SEQ ID NO: 98 - protein, 107 aa, Artificial Sequence
  hu179VL2-Y50E
DIVMTQSPDSLAVSLGERATINCKASQSVSSDVTWYQQKPGQSPKLLIYEVSNHYTGVPDRFSGSGSGTDFTLTISSLQAEDVAVYYCQQHHRFPLTFGQGTKLEIK

SEQ ID NO: 99 - protein, 107 aa, Artificial Sequence
  hu179VL2-S52D
DIVMTQSPDSLAVSLGERATINCKASQSVSSDVTWYQQKPGQSPKLLIYYVDNHYTGVPDRFSGSGSGTDFTLTISSLQAEDVAVYYCQQHHRFPLTFGQGTKLEIK

SEQ ID NO: 100 - protein, 107 aa, Artificial Sequence
  hu179VL2-S52E
DIVMTQSPDSLAVSLGERATINCKASQSVSSDVTWYQQKPGQSPKLLIYYVENHYTGVPDRFSGSGSGTDFTLTISSLQAEDVAVYYCQQHHRFPLTFGQGTKLEIK

SEQ ID NO: 101 - protein, 107 aa, Artificial Sequence
  hu179VL2-N53Q
DIVMTQSPDSLAVSLGERATINCKASQSVSSDVTWYQQKPGQSPKLLIYYVSQHYTGVPDRFSGSGSGTDFTLTISSLQAEDVAVYYCQQHHRFPLTFGQGTKLEIK

SEQ ID NO: 102 - protein, 107 aa, Artificial Sequence
  hu179VL2-N53D
DIVMTQSPDSLAVSLGERATINCKASQSVSSDVTWYQQKPGQSPKLLIYYVSDHYTGVPDRFSGSGSGTDFTLTISSLQAEDVAVYYCQQHHRFPLTFGQGTKLEIK

SEQ ID NO: 103 - protein, 107 aa, Artificial Sequence
  hu179VL2-N53E
DIVMTQSPDSLAVSLGERATINCKASQSVSSDVTWYQQKPGQSPKLLIYYVSEHYTGVPDRFSGSGSGTDFTLTISSLQAEDVAVYYCQQHHRFPLTFGQGTKLEIK

SEQ ID NO: 104 - protein, 107 aa, Artificial Sequence
  hu179VL2-H54Y
DIVMTQSPDSLAVSLGERATINCKASQSVSSDVTWYQQKPGQSPKLLIYYVSNYYTGVPDRFSGSGSGTDFTLTISSLQAEDVAVYYCQQHHRFPLTFGQGTKLEIK

SEQ ID NO: 105 - protein, 107 aa, Artificial Sequence
  hu179VL2-H54D
DIVMTQSPDSLAVSLGERATINCKASQSVSSDVTWYQQKPGQSPKLLIYYVSNDYTGVPDRFSGSGSGTDFTLTISSLQAEDVAVYYCQQHHRFPLTFGQGTKLEIK

SEQ ID NO: 106 - protein, 107 aa, Artificial Sequence
  hu179VL2-H54E
DIVMTQSPDSLAVSLGERATINCKASQSVSSDVTWYQQKPGQSPKLLIYYVSNEYTGVPDRFSGSGSGTDFTLTISSLQAEDVAVYYCQQHHRFPLTFGQGTKLEIK

SEQ ID NO: 107 - protein, 107 aa, Artificial Sequence
  hu179VL2-Y55E
DIVMTQSPDSLAVSLGERATINCKASQSVSSDVTWYQQKPGQSPKLLIYYVSNHETGVPDRFSGSGSGTDFTLTISSLQAEDVAVYYCQQHHRFPLTFGQGTKLEIK

SEQ ID NO: 108 - protein, 7 aa, Artificial Sequence
  hu179 LCDR2-Y50E
EVSNHYT

SEQ ID NO: 109 - protein, 7 aa, Artificial Sequence
  hu179 LCDR2-S52D
YVDNHYT

SEQ ID NO: 110 - protein, 7 aa, Artificial Sequence
  hu179 LCDR2-S52E
YVENHYT

SEQ ID NO: 111 - protein, 7 aa, Artificial Sequence
  hu179LCDR2-N53Q
YVSQHYT

SEQ ID NO: 112 - protein, 7 aa, Artificial Sequence
  hu179 LCDR2-N53D
YVSDHYT

SEQ ID NO: 113 - protein, 7 aa, Artificial Sequence
  hu179 LCDR2-N53E
YVSEHYT

SEQ ID NO: 114 - protein, 7 aa, Artificial Sequence
  hu179 LCDR2-H54Y
YVSNYYT

SEQ ID NO: 115 - protein, 7 aa, Artificial Sequence
  hu179 LCDR2-H54D
YVSNDYT

SEQ ID NO: 116 - protein, 7 aa, Artificial Sequence
  hu179 LCDR2-H54E
YVSNEYT

SEQ ID NO: 117 - protein, 7 aa, Artificial Sequence
  hu179 LCDR2-Y55E
YVSNHET

SEQ ID NO: 118 - protein, 7 aa, Artificial Sequence
  mab179LCDR2
  DOMAIN (1)..(1): Xaa is selected from the group consisting of Try and Glu
  DOMAIN (3)..(3): Xaa is selected from the group consisting of Ser, Asp, and Glu
  DOMAIN (4)..(4): Xaa is selected from the group consisting of Asn, Gln, Asp, and Glu
  DOMAIN (5)..(5): Xaa is selected from the group consisting of His, Tyr, Asp, and Glu
  DOMAIN (6)..(6): Xaa is selected from the group consisting of Glu and Tyr
XVXXXXT

SEQ ID NO: 119 - protein, 107 aa, Artificial Sequence
  hu179VL8-N53E
SIVMTQTPLSLSVTPGQPASISCKASQSVSSDVTWYLQKPGQSPQLLIYYVSEHYTGVPDRFSGSGYGTDFTLKISRVEAEDVGVYYCQQHHRFPLTFGQGTKLEIK

SEQ ID NO: 120 - protein, 107 aa, Artificial Sequence
  hu199VL1Grafted
DIQMTQSPSSLSASVGDRVTITCRASENIYSYLAWYQQKPGKAPKLLIYFAKTLAEGVPSRFSGSGSGTDFTLTISSLQPEDFATYYCQHHYGTPWTFGGGTKVEIK

SEQ ID NO: 121 - protein, 107 aa, Artificial Sequence
  hu199VL2
DIQMTQSPSSLSASVGDRVTITCRASENIYSYLAWYQQKPGKAPKLLVYFAKTLAEGVPSRFSGSGSGTDFTLTISSLQPEDFATYYCQHHYGTPWTFGGGTKVEIK

SEQ ID NO: 122 - protein, 107 aa, Artificial Sequence
  hu199VL3
DIQMTQSPSSLSASVGDRVTITCRASENIYSYLAWYQQKPGKSPQLLVYFAKTLAEGVPSRFSGSGSGTQFTLTISSLQPEDFATYYCQHHYGTPWTFGGGTKVEIK

SEQ ID NO: 123 - protein, 107 aa, Artificial Sequence
  hu199VL4
DIQMTQSPSSLSASVGDRVTITCRASENIYSYLAWYQQKPGKAPKLLIYFAKTLAEGVPSRFSGSVSGTDFTLTISSLQPEDFATYYCQHHYGTPWTFGGGTKVEIK

SEQ ID NO: 124 - protein, 107 aa, Artificial Sequence
  hu199VL5
DIQMTQSPSSLSASVGDRVTITCRASENIYSYLAWYQQKPGKAPKLLVYFAKTLAEGVPSRFSGSVSGTDFTLTISSLQPEDFATYYCQHHYGTPWTFGGGTKVEIK

SEQ ID NO: 125 - protein, 107 aa, Artificial Sequence
  hu199VL6
DIQMTQSPSSLSASVGDRVTITCRASENIYSYLAWYQQKPGKSPQLLVYFAKTLAEGVPSRFSGSVSGTQFTLTISSLQPEDFATYYCQHHYGTPWTFGGGTKVEIK

SEQ ID NO: 126 - protein, 117 aa, Artificial Sequence
  hu199VH1( Grafted)
EVQLVQSGAEVKKPGASVKVSCKASGYTFTTYWMHWVRQAPGQGLEWMGMIDPSDSETTLIQKFKDRVTMTRDTSTSTVYMELSSLRSEDTAVYYCARTLDGYYDYWGQGTTVTVSS

SEQ ID NO: 127 - protein, 117 aa, Artificial Sequence
  hu199VH2
EVQLVQSGAEVKKPGASVKVSCKASGYTFTTYWMHWVRQAPGQGLEWMGMIDPSDSETTLIQKFKDRVTMTVDKSTSTAYMELSSLRSEDTAVYYCARTLDGYYDYWGQGTTVTVSS

SEQ ID NO: 128 - protein, 117 aa, Artificial Sequence
  hu199VH3
EVQLVQSGAEVKKPGASVKVSCKASGYTFTTYWMHWVRQAPGQGLEWMGMIDPSDSETTLIQKFKDRVTLTVDKSTSTAYMELSSLRSEDTAVYYCARTLDGYYDYWGQGTTVTVSS

SEQ ID NO: 129 - protein, 117 aa, Artificial Sequence
  hu199VH4
EVQLVQSGAEVKKPGASVKVSCKASGYTFTTYWMHWVRQAPGQGLEWIGMIDPSDSETTLIQKFKDRATLTVDKSTSTAYMELSSLRSEDTAVYYCARTLDGYYDYWGQGTTVTVSS

SEQ ID NO: 130 - protein, 117 aa, Artificial Sequence
  hu199VH5
EVQLVQSGAEVKKPGASVKVSCKASGYTFTTYWMHWVKQAPGQGLEWIGMIDPSDSETTLIQKFKDKATLTVDKSTSTAYMELSSLRSEDTAVYYCARTLDGYYDYWGQGTTVTVSS

SEQ ID NO: 131 - protein, 117 aa, Artificial Sequence
  hu199VH6
EVQLVQSGAEVKKPGASVKVSCKASGYTFTTYWMHWVKQAPGQGLEWMGMIDPSDSETTLIQKFKDKVTMTVDKSTSTAYMELSSLRSEDTAVYYCARTLDGYYDYWGQGTTVTVSS

SEQ ID NO: 132 - protein, 117 aa, Artificial Sequence
  hu199VH7
EVQLVQSGAEVKKPGASVKVSCKASGYTFTTYWMHWVKQAPGQGLEWMGMIDPSDSETTLIQKFKDKVTLTVDKSTSTAYMELSSLRSEDTAVYYCARTLDGYYDYWGQGTTVTVSS

SEQ ID NO: 133 - protein, 330 aa, Artificial Sequence
  IgG1-YTE
ASTKGPSVFPLAPSSKSTSGGTAALGCLVKDYFPEPVTVSWNSGALTSGVHTFPAVLQSSGLYSLSSVVTVPSSSLGTQTYICNVNHKPSNTKVDKKVEPKSCDKTHTCPPCPAPELLGGPSVFLFPPKPKDTLYITREPEVTCVVVDVSHEDPEVKFNWYVDGVEVHNAKTKPREEQYNSTYRVVSVLTVLHQDWLNGKEYKCKVSNKALPAPIEKTISKAKGQPREPQVYTLPPSRDELTKNQVSLTCLVKGFYPSDIAVEWESNGQPENNYKTTPPVLDSDGSFFLYSKLTVDKSRWQQGNVFSCSVMHEALHNHYTQKSLSLSPGK

SEQ ID NO: 134 - protein, 107 aa, Artificial Sequence [sequence omitted]

SEQ ID NO: 135 - protein, 451 aa, Artificial Sequence
  hu3-13
EVQLVQSGAEVKKPGASVKVSCKASGYTFTDDYMNWVRQAPGQRLEWMGIISPYNGGTSYNQKFKGRVTLTVDKSASTAYMELSSLRSEDTAVYYCAREDYDYDGYAMDYWGQGTTVTVSSASTKGPSVFPLAPSSKSTSGGTAALGCLVKDYFPEPVTVSWNSGALTSGVHTFPAVLQSSGLYSLSSVVTVPSSSLGTQTYICNVNHKPSNTKVDKKVEPKSCDKTHTCPPCPAPELLGGPSVFLFPPKPKDTLYITREPEVTCVVVDVSHEDPEVKFNWYVDGVEVHNAKTKPREEQYNSTYRVVSVLTVLHQDWLNGKEYKCKVSNKALPAPIEKTISKAKGQPREPQVYTLPPSRDELTKNQVSLTCLVKGFYPSDIAVEWESNGQPENNYKTTPPVLDSDGSFFLYSKLTVDKSRWQQGNVFSCSVMHEALHNHYTQKSLSLSPGK

SEQ ID NO: 136 - protein, 212 aa, Artificial Sequence
  hu3-13
EIVLTQSPATLSLSPGERATLSCRASSSVSYMHWYQQKPGQAPRPWIYATSNLASGVPARFSGSGSGTSYTLTISRLEPEDFAVYYCQQSDSGREFGGGTKVEIKRTVAAPSVFIFPPSDEQLKSGTASVVCLLNNFYPREAKVQWKVDNALQSGNSQESVTEQDSKDSTYSLSSTLTLSKADYEKHKVYACEVTHQGLSSPVTKSFNRGEC

SEQ ID NO: 137 - protein, 450 aa, Artificial Sequence
  hu119-30
EAQLVQSGAEVKKPGSSVKVSCKASGFTFSTYNMHWVRQAPGQGLEWIGAIYPGNGETSYNQKFKDRATLTVDKSTRTAYMELSSLRSEDTAVYYCAREDDYGEGYFDVWGQGTTVTVSSASTKGPSVFPLAPSSKSTSGGTAALGCLVKDYFPEPVTVSWNSGALTSGVHTFPAVLQSSGLYSLSSVVTVPSSSLGTQTYICNVNHKPSNTKVDKKVEPKSCDKTHTCPPCPAPELLGGPSVFLFPPKPKDTLYITREPEVTCVVVDVSHEDPEVKFNWYVDGVEVHNAKTKPREEQYNSTYRVVSVLTVLHQDWLNGKEYKCKVSNKALPAPIEKTISKAKGQPREPQVYTLPPSRDELTKNQVSLTCLVKGFYPSDIAVEWESNGQPENNYKTTPPVLDSDGSFFLYSKLTVDKSRWQQGNVFSCSVMHEALHNHYTQKSLSLSPGK

SEQ ID NO: 138 - protein, 218 aa, Artificial Sequence
  hu119-30
DIVLTQSPATLSLSPGERATLSCRASESVDSSGLSFMHWYQQKPGQPPRLLLYRASNLGSGIPARFSGSGSGTDFTLTISSLEPEDFAVYYCQQINTDPLTFGQGTKLEIKRTVAAPSVFIFPPSDEQLKSGTASVVCLLNNFYPREAKVQWKVDNALQSGNSQESVTEQDSKDSTYSLSSTLTLSKADYEKHKVYACEVTHQGLSSPVTKSFNRGEC

SEQ ID NO: 139 - protein, 449 aa, Artificial Sequence
  hu179-33
EVQLVQSGAEVKKPGSSVKVSCKASGYTFSNYLIEWVRQAPGQGLEWIGVIDPGVGDTNYNENFKGRATLTADKSTSTAYIELSSLRSEDTAVYYCAREDNTGTAFDYWGQGTTVTVSSASTKGPSVFPLAPSSKSTSGGTAALGCLVKDYFPEPVTVSWNSGALTSGVHTFPAVLQSSGLYSLSSVVTVPSSSLGTQTYICNVNHKPSNTKVDKKVEPKSCDKTHTCPPCPAPELLGGPSVFLFPPKPKDTLYITREPEVTCVVVDVSHEDPEVKFNWYVDGVEVHNAKTKPREEQYNSTYRVVSVLTVLHQDWLNGKEYKCKVSNKALPAPIEKTISKAKGQPREPQVYTLPPSRDELTKNQVSLTCLVKGFYPSDIAVEWESNGQPENNYKTTPPVLDSDGSFFLYSKLTVDKSRWQQGNVFSCSVMHEALHNHYTQKSLSLSPGK

SEQ ID NO: 140 - protein, 214 aa, Artificial Sequence
  hu179-33
SIVMTQTPLSLSVTPGQPASISCKASQSVSSDVTWYLQKPGQSPQLLIYYVSEHYTGVPDRFSGSGYGTDFTLKISRVEAEDVGVYYCQQHHRFPLTFGQGTKLEIKRTVAAPSVFIFPPSDEQLKSGTASVVCLLNNFYPREAKVQWKVDNALQSGNSQESVTEQDSKDSTYSLSSTLTLSKADYEKHKVYACEVTHQGLSSPVTKSFNRGEC

SEQ ID NO: 141 - protein, 447 aa, Artificial Sequence
  hu199-36
EVQLVQSGAEVKKPGASVKVSCKASGYTFTTYWMHWVKQAPGQGLEWMGMIDPSDSETTLIQKFKDKVTLTVDKSTSTAYMELSSLRSEDTAVYYCARTLDGYYDYWGQGTTVTVSSASTKGPSVFPLAPSSKSTSGGTAALGCLVKDYFPEPVTVSWNSGALTSGVHTFPAVLQSSGLYSLSSVVTVPSSSLGTQTYICNVNHKPSNTKVDKKVEPKSCDKTHTCPPCPAPELLGGPSVFLFPPKPKDTLYITREPEVTCVVVDVSHEDPEVKFNWYVDGVEVHNAKTKPREEQYNSTYRVVSVLTVLHQDWLNGKEYKCKVSNKALPAPIEKTISKAKGQPREPQVYTLPPSRDELTKNQVSLTCLVKGFYPSDIAVEWESNGQPENNYKTTPPVLDSDGSFFLYSKLTVDKSRWQQGNVFSCSVMHEALHNHYTQKSLSLSPGK

SEQ ID NO: 142 - protein, 214 aa, Artificial Sequence
  hu199-36
DIQMTQSPSSLSASVGDRVTITCRASENIYSYLAWYQQKPGKSPQLLVYFAKTLAEGVPSRFSGSVSGTQFTLTISSLQPEDFATYYCQHHYGTPWTFGGGTKVEIKRTVAAPSVFIFPPSDEQLKSGTASVVCLLNNFYPREAKVQWKVDNALQSGNSQESVTEQDSKDSTYSLSSTLTLSKADYEKHKVYACEVTHQGLSSPVTKSFNRGEC

SEQ ID NO: 143 - protein, 448 aa, Artificial Sequence
  AMG157
QMQLVESGGGVVQPGRSLRLSCAASGFTFRTYGMHWVRQAPGKGLEWVAVIWYDGSNKHYADSVKGRFTITRDNSKNTLNLQMNSLRAEDTAVYYCARAPQWELVHEAFDIWGQGTMVTVSSASTKGPSVFPLAPCSRSTSESTAALGCLVKDYFPEPVTVSWNSGALTSGVHTFPAVLQSSGLYSLSSVVTVPSSNFGTQTYTCNVDHKPSNTKVDKTVERKCCVECPPCPAPPVAGPSVFLFPPKPKDTLMISRTPEVTCVVVDVSHEDPEVQFNWYVDGVEVHNAKTKPREEQFNSTFRVVSVLTVVHQDWLNGKEYKCKVSNKGLPAPIEKTISKTKGQPREPQVYTLPPSREEMTKNQVSLTCLVKGFYPSDIAVEWESNGQPENNYKTTPPMLDSDGSFFLYSKLTVDKSRWQQGNVFSCSVMHEALHNHYTQKSLSLSPGK

SEQ ID NO: 144 - protein, 214 aa, Artificial Sequence
  AMG157
SYVLTQPPSVSVAPGQTARITCGGNNLGSKSVHWYQQKPGQAPVLVVYDDSDRPSWIPERFSGSNSGNTATLTISRGEAGDEADYYCQVWDSSSDHVVFGGGTKLTVLGQPKAAPSVTLFPPSSEELQANKATLVCLISDFYPGAVTVAWKADSSPVKAGVETTTPSKQSNNKYAASSYLSLTPEQWKSHRSYSCQVTHEGSTVEKTVAPTECS

SEQ ID NO: 145 - protein, 371 aa, Artificial Sequence
  TSLP
MGRLVLLWGAAVFLLGGWMALGQGGAAEGVQIQIIYFNLETVQVTWNASKYSRTNLTFHYRFNGDEAYDQCTNYLLQEGHTSGCLLDAEQRDDILYFSIRNGTHPVFTASRWMVYYLKPSSPKHVRFSWHQDAVTVTCSDLSYGDLLYEVQYRSPFDTEWQSKQENTCNVTIEGLDAEKCYSFWVRVKAMEDVYGPDTYPSDWSEVTCWQRGEIRDACAETPTPPKPKLSKFILISSLAILLMVSLLLLSLWKLWRVKKFLIPSVPDPKSIFPGLFEIHQGNFQEWITDTQNVAHLHKMAGAEQESGPEEPLVVQLAKTEAESPRMLDPQTEEKEASGGSLQLPHQPLQGGDVVTIGGFTFVMNDRSYVAL

SEQ ID NO: 146 - protein, 459 aa, Artificial Sequence [sequence omitted]